European Patent Application EP 4 480 962 A1, published December 25, 2024. Title: LONG-ACTING GLP-1/GLP-2 DUAL AGONIST COMPOUND. Applicant: CHENGDU AODA BIOTECHNOLOGY CO., LTD. Application CN PCT/CN2022/136262, filed December 2, 2022. The sequence listing filed with the application follows.

SEQUENCE LISTING (13 sequences)

SEQ ID NO: 1 - protein, 33 aa, synthetic construct
  MOD_RES 2: note = X is Aib
  MOD_RES 16: note = gamma Glu octadecandioic acid modified lysine
  MOD_RES 33: note = -NH2 modified aspartic acid
HXEGSFTSELATILDKQAARDFIAWLIQHKITD

SEQ ID NO: 2 - protein, 33 aa, synthetic construct; identical to SEQ ID NO: 1
  MOD_RES 2: note = X=Aib
  MOD_RES 16: note = PEG1CH2CO gamma Glu octadecanedioic acid modified lysine
  MOD_RES 33: note = -NH2 modified aspartic acid

SEQ ID NO: 3 - protein, 33 aa, synthetic construct; identical to SEQ ID NO: 1
  MOD_RES 2: note = X=Aib
  MOD_RES 16: note = AEEA gamma Glu octadecanedioic acid modified lysine
  MOD_RES 33: note = -NH2 modified aspartic acid

SEQ ID NO: 4 - protein, 33 aa, synthetic construct; identical to SEQ ID NO: 1
  MOD_RES 2: note = X=Aib
  MOD_RES 16: note = PEG3CH2CO gamma Glu octadecandioic acid modified lysine
  MOD_RES 33: note = -NH2 modified aspartic acid

SEQ ID NO: 5 - protein, 33 aa, synthetic construct; identical to SEQ ID NO: 1
  MOD_RES 16: note = PEG4CH2CO gamma Glu octadecanedioic acid modified lysine
  MOD_RES 2: note = X=Aib
  MOD_RES 33: note = -NH2 modified aspartic acid

SEQ ID NO: 6 - protein, 33 aa, synthetic construct; identical to SEQ ID NO: 1
  MOD_RES 2: note = X=Aib
  MOD_RES 16: note = PEG5CH2CO gamma Glu octadecanedioic acid modified lysine
  MOD_RES 33: note = -NH2 modified aspartic acid

SEQ ID NO: 7 - protein, 33 aa, synthetic construct
  MOD_RES 2: note = X=Aib
  MOD_RES 16: note = PEG3CH2CO gamma Glu octadecandioic acid modified lysine
  MOD_RES 33: note = -NH2 modified aspartic acid
HXEGSXTSELATILDKQAARDFIAWLIQHKITD

SEQ ID NO: 8 - protein, 33 aa, synthetic construct; identical to SEQ ID NO: 7
  MOD_RES 2: note = X=Aib
  MOD_RES 6: note = X=alpha MePhe(2F)
  MOD_RES 16: note = PEG3CH2CO gamma Glu octadecandioic acid modified lysine
  MOD_RES 33: note = -NH2 modified aspartic acid

SEQ ID NO: 9 - protein, 33 aa, synthetic construct
  MOD_RES 2: note = X=Aib
  MOD_RES 6: note = X=alpha MePhe
  MOD_RES 16: note = PEG3CH2CO gamma Glu octadecandioic acid modified lysine
  MOD_RES 33: note = -NH2 modified aspartic acid
  MOD_RES 13: note = X=Aib
HXEGSXTSELATXLDKQAARDFIAWLIQHKITD

SEQ ID NO: 10 - protein, 33 aa, synthetic construct; identical to SEQ ID NO: 9
  MOD_RES 2: note = X=Aib
  MOD_RES 6: note = X=alpha-MePhe(2F)
  MOD_RES 13: note = X=Aib
  MOD_RES 16: note = PEG3CH2CO gamma Glu octadecandioic acid modified lysine
  MOD_RES 33: note = -NH2 modified aspartic acid

SEQ ID NO: 11 - protein, 33 aa, synthetic construct; identical to SEQ ID NO: 9
  MOD_RES 2: note = X=Aib
  MOD_RES 6: note = X=alpha-MePhe
  MOD_RES 13: note = X=alpha-MeLeu
  MOD_RES 16: note = PEG3CH2CO gamma Glu octadecandioic acid modified lysine
  MOD_RES 33: note = -NH2 modified aspartic acid

SEQ ID NO: 12 - protein, 33 aa, synthetic construct; identical to SEQ ID NO: 9
  MOD_RES 2: note = X=Aib
  MOD_RES 6: note = X=alpha MePhe(2F)
  MOD_RES 13: note = X=alpha MeLeu
  MOD_RES 16: note = PEG3CH2CO gamma Glu octadecandioic acid modified lysine
  MOD_RES 33: note = -NH2 modified aspartic acid

SEQ ID NO: 13 - protein, 33 aa, synthetic construct
  MOD_RES 2: note = X is Aib, Gly, Acpr, Acp, Acpe, or Ach
  MOD_RES 5: note = X is Ser or Thr
  MOD_RES 6: note = x is Phe, alpha-MePhe, or alpha-MePhe(2F)
  MOD_RES 7: note = X is Ser or Thr
  MOD_RES 13: note = X is Ile, Aib, or alpha-MeLeu
  MOD_RES 16: note = x is selected from the group consisting of Lys, Dap, Dab, Orn, Dah, Dao, Asp[NH(CH2)mNH], Glu[NH(CH2)mNH], Ada[NH(CH2)mNH], Apm[NH(CH2)mNH], and Asu[NH(CH2)mNH]; wherein: m is an integer selected from 2 to 10;; note = X is modified by R, and R is HO2C(CH2)n1CO-(AA11)n2-(PEGn3(CH2)n4CO)n5-; wherein: R is not HO2C(CH2)n1CO-(AA11)n2-(PEG2CH2CO)2-; n1 is an integer selected from 10 to 20; n2 is an integer selected from 1 to 5; n3 is an integer selected from 1 to 30; n4 is an integer selected from 1 to 5; n5 is an integer selected from 1 to 5; n6 is an integer selected from 1 to 10;
  MOD_RES 17: note = X is Gln, Glu, or Leu;
  MOD_RES 27: note = X is Ala or Gln
  MOD_RES 28: note = X is His or Thr
  MOD_RES 33: note = Aspartic acid modified with -NH2 or aspartic acid modified with -OH
HXEGXXXSELATXLDXXAARDFIAWLIXXKITD